European Patent Specification EP 3 995 139 B1, published February 18, 2026. Title: METHODS FOR TREATING CANCER AND INHIBITING GRAFT REJECTION. Applicant: Georgia State University Research Foundation, Inc. The sequence listing filed with the application follows.

SEQUENCE LISTING (12 sequences)

SEQ ID NO: 1 - RNA, 23 nt, Artificial Sequence
  Synthetic Construct
caaagugcuuacagugcagguag

SEQ ID NO: 2 - RNA, 23 nt, Artificial Sequence
  Synthetic Construct
uaaagugcuuauagugcagguag

SEQ ID NO: 3 - RNA, 23 nt, Artificial Sequence
  Synthetic Construct
aaaagugcuuacagugcagguag

SEQ ID NO: 4 - RNA, 23 nt, Artificial Sequence
  Synthetic Construct
cuaccugcacuguaagcacuuug

SEQ ID NO: 5 - RNA, 23 nt, Artificial Sequence
  Synthetic Construct
cuaccugcacuauaagcacuuua

SEQ ID NO: 6 - RNA, 23 nt, Artificial Sequence
  Synthetic Construct
cuaccugcacuguaagcacuuuu

SEQ ID NO: 7 - DNA, 24 bp, Artificial Sequence
  Synthetic Construct
ctgaaggtgactcagcctgagaaa

SEQ ID NO: 8 - DNA, 24 bp, Artificial Sequence
  Synthetic Construct
actgatacggatggaaaagtccat

SEQ ID NO: 9 - DNA, 24 bp, Artificial Sequence
  Synthetic Construct
ttgccggtgggacccattaggtgg

SEQ ID NO: 10 - DNA, 24 bp, Artificial Sequence
  Synthetic Construct
agattgtatttctgtgtcaggctc

SEQ ID NO: 11 - DNA, 20 bp, Artificial Sequence
  Synthetic Construct
tgtgctcgacgttgtcactg

SEQ ID NO: 12 - DNA, 24 bp, Artificial Sequence
  Synthetic Construct
cgataccgtaaagcacgaggaagc